European Patent Specification EP 3 097 211 B1, published September 13, 2023. Title: Method and System for Microbiome Analysis. The sequence listing filed with the application follows.

SEQUENCE LISTING (269 sequences)

SEQ ID NO: 1 - DNA, 20 bp, Degenerate Sequence
ccagcascygcggtaattcc

SEQ ID NO: 2 - DNA, 18 bp, Degenerate Sequence
actttcgttcttgatyra

SEQ ID NO: 3 - DNA, 19 bp, Primer Sequence
ccagcagctgcggtaattc

SEQ ID NO: 4 - DNA, 16 bp, Synthetic Barcode Sequence
tacgacggtacacagt

SEQ ID NO: 5 - DNA, 18 bp, Primer Sequence
tcgatcaagaacgaaagt

SEQ ID NO: 6 - DNA, 20 bp, Primer Sequence
tggtcatttagaggaagtaa

SEQ ID NO: 7 - DNA, 18 bp, Primer Sequence
tgcgttcttcatcgatgc

SEQ ID NO: 8 - DNA, 20 bp, Primer Sequence
tggtcatttagaggaagtaa

SEQ ID NO: 9 - DNA, 16 bp, Synthetic Barcode Sequence
tccgaaagggctttga

SEQ ID NO: 10 - DNA, 18 bp, Primer Sequence
gcatcgatgaagaacgca

SEQ ID NO: 11 - DNA, 19 bp, Degenerate Sequence
gtgccagcmgccgcggtaa

SEQ ID NO: 12 - DNA, 20 bp, Degenerate Sequence
ggactachvgggtwtctaat

SEQ ID NO: 13 - DNA, 20 bp, Primer Sequence
agagtttgatcctggctcag

SEQ ID NO: 14 - DNA, 17 bp, Primer Sequence
attaccgcggctgctgg

SEQ ID NO: 15 - DNA, 20 bp, Primer Sequence
agagtttgatcctggctcag

SEQ ID NO: 16 - DNA, 15 bp, Synthetic Barcode Sequence
acccgtacttctagt

SEQ ID NO: 17 - DNA, 17 bp, Primer Sequence
ccagcagccgcggtaat

SEQ ID NO: 18 - DNA, 23 bp, Fungal Primer Sequence
cttggtcatttagaggaaagtaa

SEQ ID NO: 19 - DNA, 20 bp, Fungal Primer Sequence
gctgcgttcttcatcgatgc

SEQ ID NO: 20 - DNA, 22 bp, Bacteria and Archea 16S Primer Sequence
tcagagtttgatcctggctcag

SEQ ID NO: 21 - DNA, 17 bp, Bacteria and Archea 16S Primer Sequence
attaccgcggctgctgg

SEQ ID NO: 22 - DNA, 22 bp, Bacteria and Archea 16S Degenerate Primer Sequence
cgtgtgccagcmgccgcggtaa

SEQ ID NO: 23 - DNA, 22 bp, Bacteria and Archea 16S Degenerate Primer Sequence
ccggactachvgggtwtctaat

SEQ ID NO: 24 - DNA, 20 bp, Eukaryote 18S Degenerate Primer Sequence
ccagcascygcggtaattcc

SEQ ID NO: 25 - DNA, 18 bp, Eukaryote 18S Degenerate Primer Sequence
actttcgttcttgatyra

SEQ ID NO: 26 - DNA, 20 bp, Eukaryotic Ribosomal 18S Primer Sequence
ccagcascygcggtaattcc

SEQ ID NO: 27 - DNA, 18 bp, Eukaryotic Ribosomal 18S Primer Sequence
actttcgttcttgatyra

SEQ ID NO: 28 - DNA, 22 bp, Fungal Ribosomal ITS Primer Sequence
cttggtcatttagaggaagtaa

SEQ ID NO: 29 - DNA, 20 bp, Fungal Ribosomal ITS Primer Sequence
gctgcgttcttcatcgatgc

SEQ ID NO: 30 - DNA, 19 bp, Bacterial Ribosomal 16S Primer Sequence
gtgccagcmgccgcggtaa

SEQ ID NO: 31 - DNA, 20 bp, Bacterial Ribosomal 16S Primer Sequence
ggactachvgggtwtctaat

SEQ ID NO: 32 - DNA, 20 bp, Bacterial Ribosomal 16S Primer Sequence
agagtttgatcctggctcag

SEQ ID NO: 33 - DNA, 17 bp, Bacterial Ribosomal 16S Primer Sequence
attaccgcggctgctgg

SEQ ID NO: 34 - DNA, 17 bp, Bacterial Ribosomal 16S Primer Sequence
cctacgggaggcagcag

SEQ ID NO: 35 - DNA, 18 bp, Bacterial Ribosomal 16S Primer Sequence
ccgtcaattcmtttragt

SEQ ID NO: 36 - DNA, 19 bp, Bacterial Ribosomal 16S Primer Sequence
caacgcgargaaccttacc

SEQ ID NO: 37 - DNA, 18 bp, Bacterial Ribosomal 16S Primer Sequence
acaacacgagctgacgac

SEQ ID NO: 38 - DNA, 13 bp, Bacterial Ribosomal 16S Primer Sequence
ggmttagataccc

SEQ ID NO: 39 - DNA, 15 bp, Bacterial Ribosomal 16S Primer Sequence
crtacthchcaggyg

SEQ ID NO: 40 - DNA, 17 bp, Bacterial Ribosomal 16S Primer Sequence
cctacgggaggcagcag

SEQ ID NO: 41 - DNA, 17 bp, Bacterial Ribosomal 16S Primer Sequence
attaccgcggctgctgg

SEQ ID NO: 42 - DNA, 30 bp, rbcLZ1/rbcL19b Plant Primer Sequence
atgtcaccacaaacagagactaaagcaagt

SEQ ID NO: 43 - DNA, 21 bp, rbcLZ1/rbcL19b Plant Primer Sequence
cttcttcaggtggaactccag

SEQ ID NO: 44 - DNA, 20 bp, rD5MITS2/rb1MITS2f Plant Primer Sequence
tcctccgcttattgatatgc

SEQ ID NO: 45 - DNA, 22 bp, rD5MITS2/rb1MITS2f Plant Primer Sequence
cgatacttggtgtgaattgcag

SEQ ID NO: 46 - DNA, 20 bp, Euphausiid 16S Primer Sequence
tttattggggcgataaaaat

SEQ ID NO: 47 - DNA, 22 bp, Euphausiid 16S Primer Sequence
tcgaggtcgyaatctttcttgt

SEQ ID NO: 48 - DNA, 20 bp, Mitochondrial 16S Primer Sequence
cccacatcaaatacccccta

SEQ ID NO: 49 - DNA, 20 bp, Mitochondrial 16S Primer Sequence
gggtcattggtggtcagaag

SEQ ID NO: 50 - DNA, 21 bp, Noto rDNA Primer Sequence
ccctatgaagcttyagacrta

SEQ ID NO: 51 - DNA, 23 bp, Noto rDNA Primer Sequence
ccttgttgatawggtctctaaaa

SEQ ID NO: 52 - DNA, 26 bp, Amphipod Nuclear 18S Primer Sequence
ctgcggttaaaaggctcgtagttgaa

SEQ ID NO: 53 - DNA, 24 bp, Amphipod Nuclear 18S Primer Sequence
actgctttragcactctgatttac

SEQ ID NO: 54 - DNA, 30 bp, Cephalopod 28S Primer Sequence
cgccgaatcccgtcgcmagtaaamggcttc

SEQ ID NO: 55 - DNA, 26 bp, Cephalopod 28S Primer Sequence
ccaagcaacccgactctcggatcgaa

SEQ ID NO: 56 - DNA, 15 bp, All Prey 16S Primer Sequence
gacgakaagacccta

SEQ ID NO: 57 - DNA, 22 bp, All Prey 16S Primer Sequence
cgctgttatccctadrgtaact

SEQ ID NO: 58 - DNA, 17 bp, Green Plants Primer Sequence
gggcaatcctgagccaa

SEQ ID NO: 59 - DNA, 22 bp, Green Plants Primer Sequence
ccattgagtctctgcacctatc

SEQ ID NO: 60 - DNA, 26 bp, Land Plants Primer Sequence
atgtcaccaccaacagagactaaagc

SEQ ID NO: 61 - DNA, 21 bp, Land Plants Primer Sequence
cttcttcaggtggaactccag

SEQ ID NO: 62 - DNA, 22 bp, Land Plants Primer Sequence
gttatgcatgaacgtaatgctc

SEQ ID NO: 63 - DNA, 21 bp, Land Plants Primer Sequence
cgcgcatggtggattcacaat

SEQ ID NO: 64 - DNA, 18 bp, Vertebrates 12S Primer Sequence
tagaacaggctcctctag

SEQ ID NO: 65 - DNA, 18 bp, Vertebrates 12S Primer Sequence
ttagataccccactatgc

SEQ ID NO: 66 - DNA, 20 bp, Chordata 16S Primer Sequence
cgagaagaccctrtggagct

SEQ ID NO: 67 - DNA, 19 bp, Chordata 16S Primer Sequence
ggattgcgctgttatccct

SEQ ID NO: 68 - DNA, 20 bp, Chordata 16S Primer Sequence
cgagaagaccctrtggagct

SEQ ID NO: 69 - DNA, 16 bp, Chordata 16S Primer Sequence
  misc_feature (4)..(4)"<223>  n is a, c, g, or t"
cctnggtcgccccaac

SEQ ID NO: 70 - DNA, 30 bp, Insecta COI Primer Sequence
agatattggaacwttatattttatttttgg

SEQ ID NO: 71 - DNA, 24 bp, Insecta COI Primer Sequence
wactaatcaattwccaaatcctcc

SEQ ID NO: 72 - DNA, 21 bp, Lumbricidae 12S Primer Sequence
tgtgtactgccgtcgtaagca

SEQ ID NO: 73 - DNA, 20 bp, Lumbricidae 12S Primer Sequence
aagagcgacgggcgatgtgt

SEQ ID NO: 74 - DNA, 22 bp, 16S Primer Sequence
ccggtctgaactcagatcacgt

SEQ ID NO: 75 - DNA, 20 bp, 16S Primer Sequence
cgcctgtttatcaaaaacat

SEQ ID NO: 76 - DNA, 20 bp, Papillomavirus Primer
cgtccmarrggawactgatc

SEQ ID NO: 77 - DNA, 20 bp, Papillomavirus Primer Sequence
gcmcagggwcataayaatgg

SEQ ID NO: 78 - DNA, 27 bp, Coronavirus Primer Sequence
gggawgggattacmcaaartgygaymg

SEQ ID NO: 79 - DNA, 24 bp, Coronavirus Primer Sequence
  misc_feature (16)..(16)"<223>  n is a, c, g, or t"
  misc_feature (19)..(19)"<223>  n is a, c, g, or t"
cccasaagwtgtaccnccnggytt

SEQ ID NO: 80 - DNA, 24 bp, Epstein Barr Virus
gktagactttgccagcytstaccc

SEQ ID NO: 81 - DNA, 24 bp, Epstein Barr Virus
gggagtcmgtgtcsccgtakatga

SEQ ID NO: 82 - DNA, 36 bp, Papillomavirus
  misc_feature (30)..(30)"<223>  n is a, c, g, or t"
gagcttataaacacagttattgaggayggngayatg

SEQ ID NO: 83 - DNA, 32 bp, Papillomavirus
  misc_feature (24)..(24)"<223>  n is a, c, g, or t"
aacagttgattgtcccagcagaynacrttrtt

SEQ ID NO: 84 - DNA, 15 bp, Enterovirus
tccggcccctgaatg

SEQ ID NO: 85 - DNA, 18 bp, Enterovirus
caccggatggccaatcca

SEQ ID NO: 86 - DNA, 20 bp, Influenza A Virus
cagattgctgactcccagca

SEQ ID NO: 87 - DNA, 23 bp, Influenza A Virus
gaccagcactggagctaggatga

SEQ ID NO: 88 - DNA, 25 bp, Adenovirus
gccgcagtggtcttacatgcacatc

SEQ ID NO: 89 - DNA, 23 bp, Adenovirus
cagcacgccgcggatgtcaaagt

SEQ ID NO: 90 - DNA, 20 bp, Cytomegalovirus
gttctctcgtctcctccgtg

SEQ ID NO: 91 - DNA, 20 bp, Cytomegalovirus
cctgtggagctcgttagagg

SEQ ID NO: 92 - DNA, 18 bp, Epstein Barr Virus
gagggtggtttggaaagc

SEQ ID NO: 93 - DNA, 22 bp, Epstein Barr Virus
aacagacaatggactcccttag

SEQ ID NO: 94 - DNA, 20 bp, Parovirus B19
gatactcaaccccatggaga

SEQ ID NO: 95 - DNA, 22 bp, Parovirus B19
gccctaacacatatgggtactt

SEQ ID NO: 96 - DNA, 23 bp, Human Herpes Virus
taagatgtatgctgaagaacgtg

SEQ ID NO: 97 - DNA, 19 bp, Human Herpes Virus 6
gcttgtcttcgtcgtttcg

SEQ ID NO: 98 - DNA, 21 bp, Influenza A Virus
cttctaaccgaggtcgaaacg

SEQ ID NO: 99 - DNA, 25 bp, Influenza A Virus
agggcattttggacaaagtcgtcta

SEQ ID NO: 100 - DNA, 21 bp, ABCCB-related Hyperinsulism Primer Sequence
cagctgagcccgagcccagac

SEQ ID NO: 101 - DNA, 23 bp, ABCCB-related Hyperinsulinism
tcctccctccctgctctcccgtc

SEQ ID NO: 102 - DNA, 26 bp, Alkaptonuria
gggaattctgtaaccggttaaataag

SEQ ID NO: 103 - DNA, 25 bp, Alkaptonuria
cttgctttaactcagccattttctc

SEQ ID NO: 104 - DNA, 22 bp, Alpha-1 Antitrypsin
caccgtgaaggtgcctatgatg

SEQ ID NO: 105 - DNA, 22 bp, Alpha-1 Antitrypsin
ggcattgcccaggtatttcatc

SEQ ID NO: 106 - DNA, 21 bp, Alpha-Mannosidosis
acgccagtgtcacctttagcc

SEQ ID NO: 107 - DNA, 20 bp, Alpha-Mannosidosis
gcacagccagacctcgcaat

SEQ ID NO: 108 - DNA, 20 bp, SLC12A6
tgaatcaagaaacccagact

SEQ ID NO: 109 - DNA, 21 bp, SLC12A6
attccatgttttcaccactac

SEQ ID NO: 110 - DNA, 22 bp, ARS1
cttttcccacgtggtggagtag

SEQ ID NO: 111 - DNA, 21 bp, ARS1
cccgcacaacaggtaaaagac

SEQ ID NO: 112 - DNA, 18 bp, Human
ctgaaggccgaggccaag

SEQ ID NO: 113 - DNA, 19 bp, Human
cctcacgggacacaagcag

SEQ ID NO: 114 - DNA, 22 bp, Human
ggtagctgcgtggctaacggag

SEQ ID NO: 115 - DNA, 25 bp, Human
ccacatacattatcatccactgtag

SEQ ID NO: 116 - DNA, 25 bp, Human
gaaaggatcatttctcccttgagtc

SEQ ID NO: 117 - DNA, 25 bp, Human
caggaacttgactccatagggaaag

SEQ ID NO: 118 - DNA, 20 bp, Human
cctgtcttgctttcctctcc

SEQ ID NO: 119 - DNA, 20 bp, Human
tcctcctctttccccagaag

SEQ ID NO: 120 - DNA, 22 bp, Human
gccccattacattccagatttg

SEQ ID NO: 121 - DNA, 20 bp, Human
ctcatacacggcagccacat

SEQ ID NO: 122 - DNA, 24 bp, Human
ctttcttttcgtaatatgcggcct

SEQ ID NO: 123 - DNA, 25 bp, Human
tcctgagaggatcaagactggaaac

SEQ ID NO: 124 - DNA, 20 bp, Human
gccacaatgcctctgaaagc

SEQ ID NO: 125 - DNA, 21 bp, Human
cttcatagcaaggccaagaac

SEQ ID NO: 126 - DNA, 21 bp, Human
cttcaaccctccaggctaaat

SEQ ID NO: 127 - DNA, 21 bp, Human
caaaactcgccactgacagaa

SEQ ID NO: 128 - DNA, 19 bp, Human
tggcactggctgtctcagg

SEQ ID NO: 129 - DNA, 20 bp, Human
gacaggacaggttgcaggac

SEQ ID NO: 130 - DNA, 22 bp, Human
cattctgtcacccttagaagcc

SEQ ID NO: 131 - DNA, 22 bp, Human
ggctatcagagtccagattccg

SEQ ID NO: 132 - DNA, 20 bp, Human
cgtacatacgtactgacgca

SEQ ID NO: 133 - DNA, 19 bp, Human
taagcaaccacctgacagg

SEQ ID NO: 134 - DNA, 25 bp, Human
gcatagcagagtacctgaaacagga

SEQ ID NO: 135 - DNA, 26 bp, Human
gacgtttgtctcactaatgagtgaac

SEQ ID NO: 136 - DNA, 20 bp, Human
cagattgtctacagggagct

SEQ ID NO: 137 - DNA, 20 bp, Human
cttggcaacaaacagatcag

SEQ ID NO: 138 - DNA, 20 bp, Human
actacatttcccaggattcc

SEQ ID NO: 139 - DNA, 20 bp, Human
tgcaggaagagtaacaatcg

SEQ ID NO: 140 - DNA, 25 bp, Human
atgcctagactcctgactacaacac

SEQ ID NO: 141 - DNA, 25 bp, Human
ctttgagtggcagtgagaaaataat

SEQ ID NO: 142 - DNA, 25 bp, Human
ctctcaaggtatatttctgacatac

SEQ ID NO: 143 - DNA, 21 bp, Human
caaggcgtatttgcttgagag

SEQ ID NO: 144 - DNA, 19 bp, Human
gccagtgtttttgcctgag

SEQ ID NO: 145 - DNA, 20 bp, Human
gactgctctcatagcatcgc

SEQ ID NO: 146 - DNA, 20 bp, Human
agttggcaccagctaaagat

SEQ ID NO: 147 - DNA, 20 bp, Human
tgtgaaccacagcagaatct

SEQ ID NO: 148 - DNA, 22 bp, Human
gtgaaggcactgataaaagagc

SEQ ID NO: 149 - DNA, 23 bp, Human
tggtagagtccctgaagtcagaa

SEQ ID NO: 150 - DNA, 28 bp, Human
tcaggcgctcagctccgtttcggtttca

SEQ ID NO: 151 - DNA, 26 bp, Human
aagcgccattggagccccgcacttcc

SEQ ID NO: 152 - DNA, 20 bp, Human
agaggctggggccaactgga

SEQ ID NO: 153 - DNA, 27 bp, Human
catactgcatgtgagagtctggagacg

SEQ ID NO: 154 - DNA, 23 bp, Human
acccaggagcccaagttcccttt

SEQ ID NO: 155 - DNA, 20 bp, Human
acagatcagcatggctaaat

SEQ ID NO: 156 - DNA, 20 bp, Human
ttggtgtttgctcaggaaga

SEQ ID NO: 157 - DNA, 20 bp, Human
ggcctacaggggtttcaaat

SEQ ID NO: 158 - DNA, 18 bp, Human
caatagggccggcttgac

SEQ ID NO: 159 - DNA, 22 bp, Human
tgcaacaattagttggaaaagc

SEQ ID NO: 160 - DNA, 20 bp, Human
agtgtggggtcgggagtgtg

SEQ ID NO: 161 - DNA, 20 bp, Human
cgggcagctctcggattctg

SEQ ID NO: 162 - DNA, 20 bp, Human
ccaaacccacctctagcaaa

SEQ ID NO: 163 - DNA, 18 bp, Human
agagctgaggcggaatgg

SEQ ID NO: 164 - DNA, 21 bp, Human
ctatgcctggttgcttagctg

SEQ ID NO: 165 - DNA, 22 bp, Human
cttcgttctacccgaatccatt

SEQ ID NO: 166 - DNA, 18 bp, Human
ctcaagcacagtggattg

SEQ ID NO: 167 - DNA, 19 bp, Human
gctctgaagaaaactctag

SEQ ID NO: 168 - DNA, 20 bp, Human
acggctgtcatcacttagac

SEQ ID NO: 169 - DNA, 20 bp, Human
ctccccttcctatgacatga

SEQ ID NO: 170 - DNA, 21 bp, Human
aagcactgcagtaccttggaa

SEQ ID NO: 171 - DNA, 24 bp, Human
tcatgtagcatttaccacagttga

SEQ ID NO: 172 - DNA, 10 bp, Human
tgcaagcgag

SEQ ID NO: 173 - DNA, 11 bp, Human
caagcctttat

SEQ ID NO: 174 - DNA, 22 bp, Human
acctttgcagggaatacagggc

SEQ ID NO: 175 - DNA, 24 bp, Human
tgtcttcctctctctaaggggttc

SEQ ID NO: 176 - DNA, 20 bp, Human
cggagatttaacggggacgt

SEQ ID NO: 177 - DNA, 20 bp, Human
tcgatttttccacccccgcc

SEQ ID NO: 178 - DNA, 20 bp, Human
cctaggtttgtgatgcctct

SEQ ID NO: 179 - DNA, 20 bp, Human
taggttcaactctctcctga

SEQ ID NO: 180 - DNA, 20 bp, Human
ccaggcagggacccaagaat

SEQ ID NO: 181 - DNA, 20 bp, Human
ccactccgcactgtccctct

SEQ ID NO: 182 - DNA, 16 bp, Human
acccaacccctcccac

SEQ ID NO: 183 - DNA, 17 bp, Human
agcttcagagaccggag

SEQ ID NO: 184 - DNA, 20 bp, Human
caaagaggtgccctatggtg

SEQ ID NO: 185 - DNA, 19 bp, Human
caatcacgcgagctctctc

SEQ ID NO: 186 - DNA, 20 bp, Human
caccgttatcccttaggtct

SEQ ID NO: 187 - DNA, 19 bp, Human
taggtcaagctctgggaca

SEQ ID NO: 188 - DNA, 21 bp, Human
cctatatggaaaacaatgtgg

SEQ ID NO: 189 - DNA, 20 bp, Human
aaggagctaacatttcaggc

SEQ ID NO: 190 - DNA, 21 bp, Human
gcgcttctctcggctccttag

SEQ ID NO: 191 - DNA, 19 bp, Human
ggctgcgctgggtgtagtg

SEQ ID NO: 192 - DNA, 20 bp, Human
cttcccctgcaatttcattt

SEQ ID NO: 193 - DNA, 20 bp, Human
ccagggaccttcctagacaa

SEQ ID NO: 194 - DNA, 20 bp, Human
ccatgacccaggagccattc

SEQ ID NO: 195 - DNA, 25 bp, Human
cgattacctcgacgactgagtaaga

SEQ ID NO: 196 - DNA, 29 bp, Human
ggtacgtggggctgcttgaagagacgctg

SEQ ID NO: 197 - DNA, 32 bp, Human
gaagatctgggtaggcagcaggtccagggagc

SEQ ID NO: 198 - DNA, 18 bp, Human
ccgaagcagggagctttg

SEQ ID NO: 199 - DNA, 18 bp, Human
cggtgcatgccttcacaa

SEQ ID NO: 200 - DNA, 18 bp, Human
ctacgcctgcccgcactg

SEQ ID NO: 201 - DNA, 19 bp, Human
ccaaggaccacaggggaca

SEQ ID NO: 202 - DNA, 21 bp, Human
cattcacctctgtgggtaagc

SEQ ID NO: 203 - DNA, 20 bp, Human
aggccttcacatttcacagc

SEQ ID NO: 204 - DNA, 20 bp, Human
agcattcctgatgccatgga

SEQ ID NO: 205 - DNA, 19 bp, Human
cttgcgaaagccttccttg

SEQ ID NO: 206 - DNA, 25 bp, Human
ggctgtgtcattttcttctcgctgg

SEQ ID NO: 207 - DNA, 23 bp, Human
tccaccaaacgtacccagacaag

SEQ ID NO: 208 - DNA, 24 bp, Human
tgtgtatgtgtctatcaacttatc

SEQ ID NO: 209 - DNA, 21 bp, Human
caacccccttactggaaacta

SEQ ID NO: 210 - DNA, 34 bp, Human
catgtgaagcttatgaatcctgcgagcgatgggg

SEQ ID NO: 211 - DNA, 32 bp, Human
accatggaattcctatggcctcttttccgcag

SEQ ID NO: 212 - DNA, 16 bp, Human
cccctgcgtggcagcc

SEQ ID NO: 213 - DNA, 22 bp, Human
gtctttcccaaccgatcctatc

SEQ ID NO: 214 - DNA, 26 bp, Human
cgtgcgaagatttgatgaacgaggtg

SEQ ID NO: 215 - DNA, 24 bp, Human
gcccttctgggtagtctctggatc

SEQ ID NO: 216 - DNA, 19 bp, Human
cactgcttaaccaaatcac

SEQ ID NO: 217 - DNA, 20 bp, Human
cagagcacagtgaaatttag

SEQ ID NO: 218 - DNA, 30 bp, Human
ccggaattcgagacgcttcatctgaaggaa

SEQ ID NO: 219 - DNA, 31 bp, Human
cccaagcttctgactcaaacacctgctggat

SEQ ID NO: 220 - DNA, 19 bp, Human
ccagccgctgattgggaag

SEQ ID NO: 221 - DNA, 19 bp, Human
gaactcagccaccatgtcc

SEQ ID NO: 222 - DNA, 19 bp, Human
ggacggtcttgggtcgcct

SEQ ID NO: 223 - DNA, 19 bp, Human
tgctccggggtcgctatca

SEQ ID NO: 224 - DNA, 22 bp, Human
ccgcagcacaagcacagataag

SEQ ID NO: 225 - DNA, 19 bp, Human
cccccgagtgacccccact

SEQ ID NO: 226 - DNA, 17 bp, Human
ggcacgagctgcccagg

SEQ ID NO: 227 - DNA, 19 bp, Human
cccaaaactccaagcctgc

SEQ ID NO: 228 - DNA, 23 bp, Human
gtcagagattcagggacacttgg

SEQ ID NO: 229 - DNA, 19 bp, Human
atgctttcagcctcacacc

SEQ ID NO: 230 - DNA, 29 bp, Human
cggtcgacgggggaccctttgtcatgaag

SEQ ID NO: 231 - DNA, 29 bp, Human
cgggatcccatttgataccagcggttgtt

SEQ ID NO: 232 - DNA, 37 bp, Human
actgaatgtcagtgcagtccaatttacaggctggagc

SEQ ID NO: 233 - DNA, 36 bp, Human
cctctgtcccatttgcaagcttcagtaactgttccc

SEQ ID NO: 234 - DNA, 20 bp, Human
tggaaccagatgtaccagca

SEQ ID NO: 235 - DNA, 20 bp, Human
gggaagagggactgatttgc

SEQ ID NO: 236 - DNA, 20 bp, Human
acgtagggcttaatagtggg

SEQ ID NO: 237 - DNA, 20 bp, Human
gtttaatgctcaaacgctcc

SEQ ID NO: 238 - DNA, 30 bp, Human
aatctcatttatatgtacttacatgccagt

SEQ ID NO: 239 - DNA, 29 bp, Human
ggttcatattcataccaaagaatgacatc

SEQ ID NO: 240 - DNA, 20 bp, Human
gctgctgggccagggctgtg

SEQ ID NO: 241 - DNA, 20 bp, Human
gcagaggcagctggcaccag

SEQ ID NO: 242 - DNA, 19 bp, Human
gccggcagagcggcggtac

SEQ ID NO: 243 - DNA, 18 bp, Human
ctggctcccgcgccttcc

SEQ ID NO: 244 - DNA, 20 bp, Human
tggctggattttgtacttac

SEQ ID NO: 245 - DNA, 20 bp, Human
accagaaagcaggatttagt

SEQ ID NO: 246 - DNA, 22 bp, Human
cataccacaggggcatcctcac

SEQ ID NO: 247 - DNA, 22 bp, Human
cagagcaggtgcgtgaggtgct

SEQ ID NO: 248 - DNA, 20 bp, Human
gctgactctgccagtgcctg

SEQ ID NO: 249 - DNA, 20 bp, Human
cagggccatcacaggtcccc

SEQ ID NO: 250 - DNA, 24 bp, Human
tggctatttttacctcctttgttt

SEQ ID NO: 251 - DNA, 20 bp, Human
agttccagatggatcccaga

SEQ ID NO: 252 - DNA, 20 bp, Human
agaacccctgactccttaga

SEQ ID NO: 253 - DNA, 18 bp, Human
gagggagaggcattcaaa

SEQ ID NO: 254 - DNA, 20 bp, Human
ttgtcttttgggctgtagca

SEQ ID NO: 255 - DNA, 26 bp, Human
tcatgacagagatcattgtactgaaa

SEQ ID NO: 256 - DNA, 29 bp, Human
tcccattgctcacaaaggtcttgtttttg

SEQ ID NO: 257 - DNA, 20 bp, Human
attcctcgcaacactgggaa

SEQ ID NO: 258 - DNA, 18 bp, Human
gacgccagagctgggtca

SEQ ID NO: 259 - DNA, 18 bp, Human
ctgcccaccgtccctctt

SEQ ID NO: 260 - DNA, 20 bp, Human
tgcctgtgacactgaactcc

SEQ ID NO: 261 - DNA, 20 bp, Human
tcctgaggcagaacttcacc

SEQ ID NO: 262 - DNA, 21 bp, Human
aaagcagatgggtttgttttg

SEQ ID NO: 263 - DNA, 18 bp, Human
ggccacgctggtagagag

SEQ ID NO: 264 - DNA, 10 bp, Microbiome 16S Primer Sequence
gtgccagcmg

SEQ ID NO: 265 - DNA, 10 bp, Microbiome 16S Primer Sequence
ggactachvg

SEQ ID NO: 266 - DNA, 17 bp, Microbiome Transposase
tcgtcggcagcgtcaga

SEQ ID NO: 267 - DNA, 17 bp, Microbiome Transposase Sequence
gtctcgtgggctcggag

SEQ ID NO: 268 - DNA, 14 bp, Microbiome Forward Index Sequence
aatgatacggcgac

SEQ ID NO: 269 - DNA, 14 bp, Microbiome Reverse Index Sequence
caagcagaagacgg